European Patent Application EP 4 523 706 A2, published March 19, 2025. Title: EXOSOMES COMPRISING THERAPEUTIC POLYPEPTIDES. Applicant: Evox Therapeutics LTD. Application EP. The sequence listing filed with the application follows.

SEQUENCE LISTING (2 sequences)

SEQ ID NO: 1 - protein, 5 aa, Mycobacterium tuberculosis
VVVHN

SEQ ID NO: 2 - protein, 6 aa, Mycobacterium tuberculosis
VVVHNC